European Patent Specification EP 3 723 488 B1, published July 30, 2025. Title: Therapeutic Bacteriocins. Applicant: Gangagen Inc. The sequence listing filed with the application follows.

SEQUENCE LISTING (30 sequences)

SEQ ID NO: 1 - DNA, 1689 bp, Artificial Sequence
  NCBI accession AF190857
atgagtggtggagacggtcgaggtccgggtaattcaggtctgggacataatggtggtcaggccagtgggaatgtgaacggtacgtctggtaaaggcggcccttcatcaggtgggggtacggatccaaacagcgggccgggctggggtacgacgcatacgcctaacggagatattcataactacaatccgggggagtttggtcacggagggaataaacccggtggcaatggcggtaacagcggcaatcatcccggtagttctggtggcagacagtcttcggccacagcgatggccttcggtctgcctgctctggctactccgggctccggggggctggctttagccgtttccggcgatgcgttgtcggcagccgttgctagtgtgctggctgccctgaaagggccgtttaagtttggtctgtgggggattgcgatctacggtgtgctgccttctgagattgcaaaagatgatccgaaaatgatgtcaaaaattatgacgtcattaccggccgatgcggtgacggagactccggcaagtactttaccactggaccaggcgacggttcgtgtcagacaacgggttgtggatgtggtgaaggatgagcggcagcatattgcggttgtcgcaggtcggccaatgagtgtccctgtggtggatgcgaaaccgacaaaacgtccgggggtattcagtgtgtcgattccgggtctcccgtctctgcaggtgagcgtaccgaaaggtgttccgacagcgaaagccccgccaaaaggcattgttgctgaaaaaggtgattcacgtccggctggttttacagccggtggtaactcccgtgaggccgttattcgtttcccgaaagagaccggacagaagccggtttatgtgtcggtgacagatgttcttaccccggcacaggtaaaacagcgtcaggaggaagaaaagcgtcgccagcaggcatgggacgccgctcatccggaagaggggctgaaaagagactatgataaagcgaaagccgagctggatgccgaagataaaaatattgcgaccttaaacagccgcattgcatcgacagagaaggcgctccccggtgcaagggctgctgttcaggaagccgataaaaaggtgaaagaggcagaggcgaataaggatgattttgtgacttataaccctcctcatgaatatggctccgggtggcaggatcaggttcgctatcttgataaggatattcagaatcagaatgcgaaattaaaagcggctcaggcatctttaaacgcaatgaatgaatccttatccagagataaggcttgcacttcccgggcgatggagagccggaaacaaaaggagaaaaaagcgaaggatgcagaaaataagttaaatgaggaaaagaaaaaacctcgcaagggagctaaagactacggccatgattatcatccagccccgaaaactgaagacataaagggactgggtgacctcaaaaaaggtacacctaaaacaccaatgcagggaggtggaggtaggcgtaaacgctggattggtgataaaggccgtaagatttatgaatgggactcccagcacggtgagcttgaagggtatcgtgccagtgatggcgaacacctcggggcatttgatcctaaaacgggtaagcaaattaaaggtccggatccgaaagggcgaaacattaaaaaatatctttaa

SEQ ID NO: 2 - protein, 562 aa, Artificial Sequence
  Amino acid sequence encoded by SEQ ID NO: 1
MSGGDGRGPGNSGLGHNGGQASGNVNGTSGKGGPSSGGGTDPNSGPGWGTTHTPNGDIHNYNPGEFGHGGNKPGGNGGNSGNHPGSSGGRQSSATAMAFGLPALATPGSGGLALAVSGDALSAAVASVLAALKGPFKFGLWGIAIYGVLPSEIAKDDPKMMSKIMTSLPADAVTETPASTLPLDQATVRVRQRVVDVVKDERQHIAVVAGRPMSVPVVDAKPTKRPGVFSVSIPGLPSLQVSVPKGVPTAKAPPKGIVAEKGDSRPAGFTAGGNSREAVIRFPKETGQKPVYVSVTDVLTPAQVKQRQEEEKRRQQAWDAAHPEEGLKRDYDKAKAELDAEDKNIATLNSRIASTEKALPGARAAVQEADKKVKEAEANKDDFVTYNPPHEYGSGWQDQVRYLDKDIQNQNAKLKAAQASLNAMNESLSRDKACTSRAMESRKQKEKKAKDAENKLNEEKKKPRKGAKDYGHDYHPAPKTEDIKGLGDLKKGTPKTPMQGGGGRRKRWIGDKGRKIYEWDSQHGELEGYRASDGEHLGAFDPKTGKQIKGPDPKGRNIKKYL

SEQ ID NO: 3 - DNA, 2298 bp, Artificial Sequence
  NCBI accession: NC_002610.1
atgggtggtggatttaactataacggggaaggtgctactggcaccggattggatcgtgatccatatgttcgcgacagcaatggtaatgctattggtgttaaatcacgctatcacgcggagtcctatgggacgtcaagtccagccttagggcctaatggcgctattcagattactgctggggttattgctgtgcctggagataagccccgacctgacggtggtagtggtggtgggaatactgttaacaccggacctgcaggacagctcctggtgatgaataaaggtcagcttggatactgggaaactcgttctacgggcgcgggtaacaatgagcataatacgagtgtatttgttgctgtaggtccttctgaggcagaaaaaactgcttctgcagagaaggcgttaaaggaaaaacagcaggcagaagcagcagcaaaagactttgcggctaaaactgctgccgcatcagccacggcggaaaaagaacgccagcaggcaattgctgctgcaactgcagcgggtcagcatcagtcagtttctgatgcccgtaatagcctgaataacgcgacgtcagatgtgtctcgtctgaaatcagctgcagacagtgcactgcaggaggcaaaggcaaaacggaaggctgctattgatgctgtacctgttgcaacccaggcggaaaataaatatcaggagctgcagcagaagattaaaggcctgaagctgaaaaatggtgagtatggtacggataaatgggaaataattggctctaataaggagcatgatcactggggatacaggttttatccatccggaattaccaaagctcaggttgatgcggcgcagatcgatgctgtgaataagcgaaatcaggctaccagtcttgccagtcaggcaacagcagcagaacaggacagcctgaaagctacagctgcctataatgcggcagaaacgcgccgtcaggctgctcaggcggcgttaaattctgctgaacaggctgctgctgctgaacgtaagcggcaggaagctgaggcggctgcagcagctgctgctgagaaaaaacgtcaggcagacgcagcagcaaaagctgcagaggaagcgcgtgcggcagcggaaaaagccaggctgatgcaggagcgtcaggcagcagcagataagctgaaatccacagatattcagtctgttcgcgggatcccgtctacggctgcgcctgcagcgtcacccatttcctgggccgttgcatcacttggtggtatatcgctggatagtgttactgcagggaaagcatggacgcagattgctgaggtgatggctaaactacgaggtattgccggtgcgagtcttgttggtcccgtggtggcaactgctgtagggctgttttggtcacgtgatgttggtattggcagtgatgtggtgcccggacgtgacatcagcgggctgatgccgggtgatgcactgtcattacctgatctggccactttgattaaagctgctgacagtaaaacgggtgtcagtatgccggttcgaggccggattatcgtgcgtgaaggcgattatctggagtctcagttcgttcgaacacctgttgccggtagtgttccggttgttcgggctgctctggataaagctactggttactggggatatacgttgccggcgatacagggtgtgcccggacagacaatactggtgagtccgtcagatgcgccgggcgttaatggtcctctgggacttgctgggccggttcctttgcctgaaactattatacataccggtgggcaaactacggttcctcagggggggactgtgacagtttcgccggcagaagacgatattgatttcaatgatttgattctggtatttccgccggagtccggtcttaaaccgttgtatgtgatgtaccgtagccctcgtaacatgccggggacagccagtggtaaaggtcagaacgttggaaataactggatgggggggaccagtaccggggatggtgctcctgttccttcccagattgcagataaattacgtgggaaggctttcggtagttttgattctttctgtcgggctttctggaaagcggttgctgctgatccggacctcagtaagcagttttatcctgatgatatagagcgaatgaaattagggcgagctccaacagttcgattccgagattctgtaggtaaaagggttaaggttgaactacaccataaagttgaaatttctaaaggtggtgatgtctataacgtagataacctgaatgcattaacacctaaacgtcatattgaaattcataaggggaactga

SEQ ID NO: 4 - protein, 765 aa, Artificial Sequence
  Amino acid sequence encoded by SEQ ID NO: 3
MGGGFNYNGEGATGTGLDRDPYVRDSNGNAIGVKSRYHAESYGTSSPALGPNGAIQITAGVIAVPGDKPRPDGGSGGGNTVNTGPAGQLLVMNKGQLGYWETRSTGAGNNEHNTSVFVAVGPSEAEKTASAEKALKEKQQAEAAAKDFAAKTAAASATAEKERQQAIAAATAAGQHQSVSDARNSLNNATSDVSRLKSAADSALQEAKAKRKAAIDAVPVATQAENKYQELQQKIKGLKLKNGEYGTDKWEIIGSNKEHDHWGYRFYPSGITKAQVDAAQIDAVNKRNQATSLASQATAAEQDSLKATAAYNAAETRRQAAQAALNSAEQAAAAERKRQEAEAAAAAAAEKKRQADAAAKAAEEARAAAEKARLMQERQAAADKLKSTDIQSVRGIPSTAAPAASPISWAVASLGGISLDSVTAGKAWTQIAEVMAKLRGIAGASLVGPVVATAVGLFWSRDVGIGSDVVPGRDISGLMPGDALSLPDLATLIKAADSKTGVSMPVRGRIIVREGDYLESQFVRTPVAGSVPVVRAALDKATGYWGYTLPAIQGVPGQTILVSPSDAPGVNGPLGLAGPVPLPETIIHTGGQTTVPQGGTVTVSPAEDDIDFNDLILVFPPESGLKPLYVMYRSPRNMPGTASGKGQNVGNNWMGGTSTGDGAPVPSQIADKLRGKAFGSFDSFCRAFWKAVAADPDLSKQFYPDDIERMKLGRAPTVRFRDSVGKRVKVELHHKVEISKGGDVYNVDNLNALTPKRHIEIHKGN

SEQ ID NO: 5 - DNA, 1855 bp, Artificial Sequence
  NCBI accession: AY578793.1
atggcagataatcaaccggttcctcttacccccgcaccacctggaatggtatcacttggcgtcaatgaaaacggcgaagaggagatgactgtcattggtggagatggcagcggcacagggttttctgggaatgaagcacctattattcctggaagtggtagcctccaggccgacttaggtaaaaagtctctaacccgactacaggctgaaagttcagcagcaattcatgcgactgcaaaatggactacagagaatcttgcaaaaacgcaggctgcgcaggctgaaagggccaaggctgccatgctttctcagcaggcagcaaaagcaaaacaggccaaactcacgctacatctgaaagatgtagtggatcgcgcgcttcagaacaacaaaacgcggcctactgttattgatcttgctcatcagaataaccaacaaatggccgcaatggccgagtttataggccgtcaaaaggcaattgaagaagctcgtaaaaaggctgaaagggaagccaaaagggctgaagaagcttatcaggctgctttgagagcgcaggaagaagaacagcgcaagcaggcagaaattgaacggaaattgcaggaggcaaggaagcaagaggcagcggcaaaagcaaaagctgaagctgacagaattgcggctgagaaagctgaagcagaggcaagagctaaagcggaagctgagcgacggaaagcagaggaggctcgaaaggcgctttttgcaaaggctgggattaaggacactcctgtttatacactggagaagacaaaagcagccactacgttgtttttaacaccgggtgttaggttactgaatcgtgctccagcgatgatacagttatccgctttggctgcagaaattaatggcgtcttaactactgctgctagtgcagtaatgacggctactgctgaattctcaggttggattgcctcagcgttatggcgaggtgtagctggtgttgcaacagctagtactgttggtcccatggttgccgcagcatcgacgctattcttttcacctcgcgcaggtggcggaagcgacagtaaggttcctggtagggatatcgagatgttggctgcgcaagccaggttgttcacggcgggtaagctgagtatcgaacatgaagagcgtcaacctcccggtacgtggcttcatctcttcggaaactgatgggcgccagtctctgatgcttgtaaaaaccggttctgatggagtaccttccactgttcctgtattggatgctgtacgtgacagtactactggccttgataaaataacggtaccggcgatgtctggtgcgccgtcgcggaccatcctcgtgaatccggttccaattggacctgctgctccgtggcataccggcaatagcgggccagtgccagtaacacctgttcacaccggtacagaggtgaagcaggctgacagtatcgtcacgacaactttgccgattgcagacattccgccactacaggacttcatctactggcagccggatgcttctgggacaggtgttgaacctatttatgtaatgactagtcaacccaggaaaggagtaaaagactacggacatgattatcatccggctccaaaaactgaagaaattaaggggttgggggagttgattgagtctcggaaaaaaactccaaaacaagggggaggtggacgacgagatcgatgggtgggagataaaggacgaaaaatctatgagtgggattcgcagcatggagaacttgaaggttacagagctagcgacggctctcatcttggagcatttgatccaaacaccggcaagcaacttaaaggtccggaccctaaacgtaacatcaaaaaatatctttga

SEQ ID NO: 6 - protein, 619 aa, Artificial Sequence
  Amino acid sequence encoded by SEQ ID NO: 5
MADNQPVPLTPAPPGMVSLGVNENGEEEMTVIGGDGSGTGFSGNEAPIIPGSGSLQADLGKKSLTRLQAESSAAIHATAKWTTENLAKTQAAQAERAKAAMLSQQAAKAKQAKLTLHLKDVVDRALQNNKTRPTVIDLAHQNNQQMAAMAEFIGRQKAIEEARKKAEREAKRAEEAYQAALRAQEEEQRKQAEIERKLQEARKQEAAAKAKAEADRIAAEKAEAEARAKAEAERRKAEEARKALFAKAGIKDTPVYTLEKTKAATTLFLTPGVRLLNRAPAMIQLSALAAEINGVLTTAASAVMTATAEFSGWIASALWRGVAGVATASTVGPMVAAASTLFFSPRAGGGSDSKVPGRDIEMLAAQARLFTAGKLSIEPGMKSVNLPVRGFISSETDGRQSLMLVKTGSDGVPSTVPVLDAVRDSTTGLDKITVPAMSGAPSRTILVNPVPIGPAAPWHTGNSGPVPVTPVHTGTEVKQADSIVTTTLPIADIPPLQDFIYWQPDASGTGVEPIYVMTSQPRKGVKDYGHDYHPAPKTEEIKGLGELIESRKKTPKQGGGGRRDRWVGDKGRKIYEWDSQHGELEGYRASDGSHLGAFDPNTGKQLKGPDPKRNIKKYL

SEQ ID NO: 7 - DNA, 2151 bp, Artificial Sequence
  NCBI accession: AY578792
atgagtgatatcacatataatcctgaggactataacaatggtataccacctgagccgggtctggtgtggaagccgggaggctcattccccaatggcagttacgttcccggctcatggggctggccaacgcgcggatacgatgttcctccgctgccgggtgataccgaaatgctgacggtcaccccaaaaggaacgccggctgatacctggcctaaaagacctgatatcaaagagtggtatgttccgggtgaaaaacccttcgacccgtcaacaggtaatggatgggtgcctgatgtggacggctacgccgaatcgctgcctgccggtataccggctgtggtacaggctgcaatcagtaaggtgaaaggtgcgccactgaaaggcggcatgtccgccgtggatatctggaaactgaaacccgcaacggagtacccggggagatttaacagcaccgacccggcattcagctggtttccggttcgggcgctgactgacactgatatatctgcgatgcccgttgcccctgagactgttccggtgcatacccgtatccttgataatgttcatgatggtgtacagtttgtttctgcggtgtttgcgggtagcatgcagtacaatctgccggtggtgaaagcgcaggccactgccggcagtgattattacactatcggacgtctgccgggcatcatgagtgctttcacattctctttctacacaaaaggaacaccacaggactcccgtttcttccgggatacagtgaaagccgggggagatttacgcgaagcaggcttcactgtgggggccaataccagcgattttatcatctggtttccgcaggggagcggactggagccgctgtatttttccatgaccatgaatatgccggctgggccgctgcagcgtcgccaggaagccgaaaacaaggccagagcagaagctgacaggctccgggcagaggcggaggcaaaaattcgcgctgaagcagaggcccgggcgaaagcagaagcagaacgcaaagccctgttcgctaaggccggtattcaggatacaccggtttacacgccggagatggtgaaggcggcaaatgcggcgctgtctgccggaggctcaatggcgctcagccgggccccggggatgatacagcactctgctgcaggcgtggggacgctacccttcaacagtagtctggcgggatgggaagccggcgcgctctggcgcggtgtcgacgtgcttgccaggatcgcgccggtcgcgtccgccgtggccacggttgccacagtgctcacccttgtcagggctgcactggatatccctgcagccggcgagggcagtgacagggttcccggacgcaacattgacatgcttgccgcccaggccagcctgtacacggccatgaagacgaacattcagccggggatgaagaccgttgacctgccagtcaggggatatatctcgtatgacggcaacggccggcagtcggtcaacttggtcaggacggggacgggcggggtttcggccacggtgccggtgctgagtgccgtgcgtgacaaaaccaccggcctggataaaatcacggtaccggccgtggcgggcgccccgtcgcggaccatcctgattaaccctgtaccggtcggtcctgcgacaccatcgcataccggcagcagtacgccggttccggtgacgccggtgcacactggtaccgatgttaagcaggcggacagcatcgtcaccacaacgttgccggcggcagatattcctgcgctgcaggacttcatctactggcagccggatgcaaccgggacgggcgtggaacccatctatgtcatgctgagtgatccgttggattcggggaaatatacccgcaggcagctccagaagaagtacaagcatgctatcgattttggtatcacagatacgaagataaatggtgaaacacttactaagttccgggatgcaattgaagcacatctttcagataaggatacctttgaaaaaggaacatatcggcgtgataagggatcgaaggtttatttcaatcctaaaacaatgaatgctgttattattcaggctaatggtgactttctgtctggatggaaaattaatcctgcggcagataatggtagaatttatttagaaacgggtgatttatga

SEQ ID NO: 8 - protein, 716 aa, Artificial Sequence
  Amino acid sequence encoded by SEQ ID NO: 7
MSDITYNPEDYNNGIPPEPGLVWKPGGSFPNGSYVPGSWGWPTRGYDVPPLPGDTEMLTVTPKGTPADTWPKRPDIKEWYVPGEKPFDPSTGNGWVPDVDGYAESLPAGIPAVVQAAISKVKGAPLKGGMSAVDIWKLKPATEYPGRFNSTDPAFSWFPVRALTDTDISAMPVAPETVPVHTRILDNVHDGVQFVSAVFAGSMQYNLPVVKAQATAGSDYYTIGRLPGIMSAFTFSFYTKGTPQDSRFFRDTVKAGGDLREAGFTVGANTSDFIIWFPQGSGLEPLYFSMTMNMPAGPLQRRQEAENKARAEADRLRAEAEAKIRAEAEARAKAEAERKALFAKAGIQDTPVYTPEMVKAANAALSAGGSMALSRAPGMIQHSAAGVGTLPFNSSLAGWEAGALWRGVDVLARIAPVASAVATVATVLTLVRAALDIPAAGEGSDRVPGRNIDMLAAQASLYTAMKTNIQPGMKTVDLPVRGYISYDGNGRQSVNLVRTGTGGVSATVPVLSAVRDKTTGLDKITVPAVAGAPSRTILINPVPVGPATPSHTGSSTPVPVTPVHTGTDVKQADSIVTTTLPAADIPALQDFIYWQPDATGTGVEPIYVMLSDPLDSGKYTRRQLQKKYKHAIDFGITDTKINGETLTKFRDAIEAHLSDKDTFEKGTYRRDKGSKVYFNPKTMNAVIIQANGDFLSGWKINPAADNGRIYLETGDL

SEQ ID NO: 9 - DNA, 1386 bp, Artificial Sequence
  DNA sequence of Klebicin CCL along with immunity gene. AF190857.1:166-1854 Klebsiella pneumoniae cloacin operon, complete sequence, 1956 bases
atgagtggtggagacggtcgaggtccgggtaattcaggtctgggacataatggtggtcaggccagtgggaatgtgaacggtacgtctggtaaaggcggcccttcatcaggtgggggtacggatccaaacagcgggccgggctggggtacgacgcatacgcctaacggagatattcataactacaatccgggggagtttggtcacggagggaataaacccggtggcaatggcggtaacagcggcaatcatcccggtagttctggtggcagacagtcttcggccacagcgatggccttcggtctgcctgctctggctactccgggctccggggggctggctttagccgtttccggcgatgcgttgtcggcagccgttgctagtgtgctggctgccctgaaagggccgtttaagaaaagagactatgataaagcgaaagccgagctggatgccgaagataaaaatattgcgaccttaaacagccgcattgcatcgacagagaaggcgctccccggtgcaagggctgctgttcaggaagccgataaaaaggtgaaagaggcagaggcgaataaggatgattttgtgacttataaccctcctcatgaatatggctccgggtggcaggatcaggttcgctatcttgataaggatattcagaatcagaatgcgaaattaaaagcggctcaggcatctttaaacgcaatgaatgaatccttatccagagataaggcttgcacttcccgggcgatggagagccggaaacaaaaggagaaaaaagcgaaggatgcagaaaataagttaaatgaggaaaagaaaaaacctcgcaagggagctaaagactacggccatgattatcatccagccccgaaaactgaagacataaagggactgggtgacctcaaaaaaggtacacctaaaacaccaatgcagggaggtggaggtaggcgtaaacgctggattggtgataaaggccgtaagatttatgaatgggactcccagcacggtgagcttgaagggtatcgtgccagtgatggcgaacacctcggggcatttgatcctaaaacgggtaagcaaattaaaggtccggatccgaaagggcgaaacattaaaaaatatctttaagaggtaagtatgggacttaaattaaatttaacctggtttgataagaaaactgaagagtttaaaggggaagagtattctaaagactttggtgatgatggttctgtcattgaaagtcttgggatgcctttaaaggataatattaacaatggttgttttgatgtgaaaaatgagtgggtttcattattgcaaccctactttaaacataaaatcaatctttctgatagttcatattttgtttcatttgattatcgggatggtaactggtaa

SEQ ID NO: 10 - protein, 562 aa, Artificial Sequence; identical to SEQ ID NO: 2
  Amino acid sequence of klebicin CCL

SEQ ID NO: 11 - DNA, 2107 bp, Artificial Sequence
  Klebicin CCL TDRD + Kleb B KD + Imm: 2107 bases
atgagtggtggagacggtcgaggtccgggtaattcaggtctgggacataatggtggtcaggccagtgggaatgtgaacggtacgtctggtaaaggcggcccttcatcaggtgggggtacggatccaaacagcgggccgggctggggtacgacgcatacgcctaacggagatattcataactacaatccgggggagtttggtcacggagggaataaacccggtggcaatggcggtaacagcggcaatcatcccggtagttctggtggcagacagtcttcggccacagcgatggccttcggtctgcctgctctggctactccgggctccggggggctggctttagccgtttccggcgatgcgttgtcggcagccgttgctagtgtgctggctgccctgaaagggccgtttaagtttggtctgtgggggattgcgatctacggtgtgctgccttctgagattgcaaaagatgatccgaaaatgatgtcaaaaattatgacgtcattaccggccgatgcggtgacggagactccggcaagtactttaccactggaccaggcgacggttcgtgtcagacaacgggttgtggatgtggtgaaggatgagcggcagcatattgcggttgtcgcaggtcggccaatgagtgtccctgtggtggatgcgaaaccgacaaaacgtccgggggtattcagtgtgtcgattccgggtctcccgtctctgcaggtgagcgtaccgaaaggtgttccgacagcgaaagccccgccaaaaggcattgttgctgaaaaaggtgattcacgtccggctggttttacagccggtggtaactcccgtgaggccgttattcgtttcccgaaagagaccggacagaagccggtttatgtgtcggtgacagatgttcttaccccggcacaggtaaaacagcgtcaggaggaagaaaagcgtcgccagcaggcatgggacgccgctcatccggaagaggggctgaaaagagactatgataaagcgaaagccgagctggatgccgaagataaaaatattgcgaccttaaacagccgcattgcatcgacagagaaggcgctccccggtgcaagggctgctgttcaggaagccgataaaaaggtgaaagaggcagaggcgaataaggatgattttgtgacttataaccctcctcatgaatatggctccgggtggcaggatcaggttcgctatcttgataaggatattcagaatcagaatgcgaaattaaaagcggctcaggcatctttaaacgcaatgaatgaatccttatccagagataaggcttgcacttcccgggcgatggagagccggaaacaaaaggagaaaaaagcgaaggatgcagaaaataagttaaatgaggaaaagaaaaaacctcgcaagggagctaaagactacggccatgatggtcttaaaccgttgtatgtgatgtaccgtagccctcgtaacatgccggggacagccagtggtaaaggtcagaacgttggaaataactggatgggggggaccagtaccggggatggtgctcctgttccttcccagattgcagataaattacgtgggaaggctttcggtagttttgattctttctgtcgggctttctggaaagcggttgctgctgatccggacctcagtaagcagttttatcctgatgatatagagcgaatgaaattagggcgagctccaacagttcgattccgagattctgtaggtaaaagggttaaggttgaactacaccataaagttgaaatttctaaaggtggtgatgtctataacgtagataacctgaatgcattaacacctaaacgtcatattgaaattcataaggggaactgaaatggctaataaaactttggctgactatacagagcaggaatttattgagtttatcgaaaaaattaaaaaggcagactttgctactgagtctgagcatgatgaggctatttatgagttcagccagttgactgagcatccagatggttgggatcttatttatcatcctcaagcaggagccgataactctcctgctggtgttgtaaaaacagtaaaagagtggcgagcagctaacggtaagccaggttttaaaaaatcgtga

SEQ ID NO: 12 - protein, 615 aa, Artificial Sequence
  Kleb CCL TD RBD (1-1419); Klebicib B KD (1420-1849); Klebicibn B Immunity protein (1850-end)
MSGGDGRGPGNSGLGHNGGQASGNVNGTSGKGGPSSGGGTDPNSGPGWGTTHTPNGDIHNYNPGEFGHGGNKPGGNGGNSGNHPGSSGGRQSSATAMAFGLPALATPGSGGLALAVSGDALSAAVASVLAALKGPFKFGLWGIAIYGVLPSEIAKDDPKMMSKIMTSLPADAVTETPASTLPLDQATVRVRQRVVDVVKDERQHIAVVAGRPMSVPVVDAKPTKRPGVFSVSIPGLPSLQVSVPKGVPTAKAPPKGIVAEKGDSRPAGFTAGGNSREAVIRFPKETGQKPVYVSVTDVLTPAQVKQRQEEEKRRQQAWDAAHPEEGLKRDYDKAKAELDAEDKNIATLNSRIASTEKALPGARAAVQEADKKVKEAEANKDDFVTYNPPHEYGSGWQDQVRYLDKDIQNQNAKLKAAQASLNAMNESLSRDKACTSRAMESRKQKEKKAKDAENKLNEEKKKPRKGAKDYGHDGLKPLYVMYRSPRNMPGTASGKGQNVGNNWMGGTSTGDGAPVPSQIADKLRGKAFGSFDSFCRAFWKAVAADPDLSKQFYPDDIERMKLGRAPTVRFRDSVGKRVKVELHHKVEISKGGDVYNVDNLNALTPKRHIEIHKGN

SEQ ID NO: 13 - DNA, 1590 bp, Artificial Sequence
  P623: S5 TD-RD-Linker-GP36 CD-his: 1590 bases
atgtccaatgacaacgaagtacctggttccatggttattgtcgcacaaggtccagacgatcaatacgcatacgaggttccccctatcgatagcgcggccgttgccgggaatatgtttggcgacttaattcaaagagaaatatatctacagaaaaacatttattatccagtccgatctatttttgaacaaggaacaaaagaaaagaaggagatcaacaagaaagtatctgatcaagtcgatggcttgctaaagcagatcactcaaggaaaaagggaggccacaaggcaagagcgagtcgatgtcatgtcggcagtcctgcacaagatggaatctgatcttgaaggatacaaaaagacctttaccaaaggcccattcattgactacgaaaagcagtcaagcctctccatctatgaggcctgggtcaagatctgggagaagaactcttgggaagaaagaaagaagtacccttttcagcagcttgttagagatgaactggagcgggcggttgcctactacaaacaagattcactctctgaagcggtaaaagtgctaagacaggagctcaacaagcaaaaagcgctaaaggaaaaagaggacctctctcaactggagcgggactacagaacccgaaaggcgaatctcgagatgaaagtacaatccgagcttgatcaagcgggaagtgctttgcctccattggtcagtccaacgccagagcaatggcttgaacgtgccacaagactggttacgcaagcaattgctgataaaaagcagctgcagaccacaaacaatactcttatcaagaattccccaacccctctagaaaagcagaaagccatctacaatggtgagctacttgtggatgagatagccagtctacaggcccgcttagttaagctgaacggaggaggaggatcaggtgtggccctggaccgcacgcgggttgatccccaggcagtcggcaacgaggtgctcaagcgcaacgcggataagctgaatgcgatgcggggcgccgagtacggtgccaacgtcaaggtcagcggcacggacattcgcatgaacgggggtaacagtgccggcatgctgaagcaggacgtgttcaactggcggaaggaactggctcagttcgaggcttaccgaggggaggcgtataaggatgccgatggttatagtgtgggcctggggcattacctgggcagtggcaatgctggggcaggtactacagtcacgcctgagcaagccgcgcagtggttcgccgaggacaccgaccgcgcactcgaccagggtgtgaggttggccgacgagctgggcgttacgaacaatgcctctatcctgggattggccggtatggccttccagatgggcgaaggacgtgcccggcagttccgtaacaccttccaggcgatcaaggatcgcaacaaggaagccttcgaggctggtgtgcgaaacagcaagtggtacacgcagacgcccaaccgggccgaggcattcatcaagcgcatggcgccccacttcgatacaccgagtcaaatcggtgtcgattggtacagcgccgcaacagcggagctcgagcaccaccaccaccaccactaa

SEQ ID NO: 14 - protein, 529 aa, Artificial Sequence
  Protein; Theoretical pI/Mw: 6.56 / 59443.77
MSNDNEVPGSMVIVAQGPDDQYAYEVPPIDSAAVAGNMFGDLIQREIYLQKNIYYPVRSIFEQGTKEKKEINKKVSDQVDGLLKQITQGKREATRQERVDVMSAVLHKMESDLEGYKKTFTKGPFIDYEKQSSLSIYEAWVKIWEKNSWEERKKYPFQQLVRDELERAVAYYKQDSLSEAVKVLRQELNKQKALKEKEDLSQLERDYRTRKANLEMKVQSELDQAGSALPPLVSPTPEQWLERATRLVTQAIADKKQLQTTNNTLIKNSPTPLEKQKAIYNGELLVDEIASLQARLVKLNGGGGSGVALDRTRVDPQAVGNEVLKRNADKLNAMRGAEYGANVKVSGTDIRMNGGNSAGMLKQDVFNWRKELAQFEAYRGEAYKDADGYSVGLGHYLGSGNAGAGTTVTPEQAAQWFAEDTDRALDQGVRLADELGVTNNASILGLAGMAFQMGEGRARQFRNTFQAIKDRNKEAFEAGVRNSKWYTQTPNRAEAFIKRMAPHFDTPSQIGVDWYSAATAELEHHHHHH

SEQ ID NO: 15 - DNA, 1566 bp, Artificial Sequence
  P624: S5 TD-RD-Link-GP36 CD without his tag: 1572 bases
atgtccaatgacaacgaagtacctggttccatggttattgtcgcacaaggtccagacgatcaatacgcatacgaggttccccctatcgatagcgcggccgttgccgggaatatgtttggcgacttaattcaaagagaaatatatctacagaaaaacatttattatccagtccgatctatttttgaacaaggaacaaaagaaaagaaggagatcaacaagaaagtatctgatcaagtcgatggcttgctaaagcagatcactcaaggaaaaagggaggccacaaggcaagagcgagtcgatgtcatgtcggcagtcctgcacaagatggaatctgatcttgaaggatacaaaaagacctttaccaaaggcccattcattgactacgaaaagcagtcaagcctctccatctatgaggcctgggtcaagatctgggagaagaactcttgggaagaaagaaagaagtacccttttcagcagcttgttagagatgaactggagcgggcggttgcctactacaaacaagattcactctctgaagcggtaaaagtgctaagacaggagctcaacaagcaaaaagcgctaaaggaaaaagaggacctctctcaactggagcgggactacagaacccgaaaggcgaatctcgagatgaaagtacaatccgagcttgatcaagcgggaagtgctttgcctccattggtcagtccaacgccagagcaatggcttgaacgtgccacaagactggttacgcaagcaattgctgataaaaagcagctgcagaccacaaacaatactcttatcaagaattccccaacccctctagaaaagcagaaagccatctacaatggtgagctacttgtggatgagatagccagtctacaggcccgcttagttaagctgaacggaggaggaggatcaggtgtggccctggaccgcacgcgggttgatccccaggcagtcggcaacgaggtgctcaagcgcaacgcggataagctgaatgcgatgcggggcgccgagtacggtgccaacgtcaaggtcagcggcacggacattcgcatgaacgggggtaacagtgccggcatgctgaagcaggacgtgttcaactggcggaaggaactggctcagttcgaggcttaccgaggggaggcgtataaggatgccgatggttatagtgtgggcctggggcattacctgggcagtggcaatgctggggcaggtactacagtcacgcctgagcaagccgcgcagtggttcgccgaggacaccgaccgcgcactcgaccagggtgtgaggttggccgacgagctgggcgttacgaacaatgcctctatcctgggattggccggtatggccttccagatgggcgaaggacgtgcccggcagttccgtaacaccttccaggcgatcaaggatcgcaacaaggaagccttcgaggctggtgtgcgaaacagcaagtggtacacgcagacgcccaaccgggccgaggcattcatcaagcgcatggcgccccacttcgatacaccgagtcaaatcggtgtcgattggtacagcgccgcaacagcggagtaa

SEQ ID NO: 16 - protein, 521 aa, Artificial Sequence
  Protein; Theoretical pI/Mw: 6.19 / 58620.92
MSNDNEVPGSMVIVAQGPDDQYAYEVPPIDSAAVAGNMFGDLIQREIYLQKNIYYPVRSIFEQGTKEKKEINKKVSDQVDGLLKQITQGKREATRQERVDVMSAVLHKMESDLEGYKKTFTKGPFIDYEKQSSLSIYEAWVKIWEKNSWEERKKYPFQQLVRDELERAVAYYKQDSLSEAVKVLRQELNKQKALKEKEDLSQLERDYRTRKANLEMKVQSELDQAGSALPPLVSPTPEQWLERATRLVTQAIADKKQLQTTNNTLIKNSPTPLEKQKAIYNGELLVDEIASLQARLVKLNGGGGSGVALDRTRVDPQAVGNEVLKRNADKLNAMRGAEYGANVKVSGTDIRMNGGNSAGMLKQDVFNWRKELAQFEAYRGEAYKDADGYSVGLGHYLGSGNAGAGTTVTPEQAAQWFAEDTDRALDQGVRLADELGVTNNASILGLAGMAFQMGEGRARQFRNTFQAIKDRNKEAFEAGVRNSKWYTQTPNRAEAFIKRMAPHFDTPSQIGVDWYSAATAE

SEQ ID NO: 17 - DNA, 1365 bp, Artificial Sequence
  P625: S5 TD-RD-Link-Phi29CD: 1365 bases
atgtccaatgacaacgaagtacctggttccatggttattgtcgcacaaggtccagacgatcaatacgcatacgaggttccccctatcgatagcgcggccgttgccgggaatatgtttggcgacttaattcaaagagaaatatatctacagaaaaacatttattatccagtccgatctatttttgaacaaggaacaaaagaaaagaaggagatcaacaagaaagtatctgatcaagtcgatggcttgctaaagcagatcactcaaggaaaaagggaggccacaaggcaagagcgagtcgatgtcatgtcggcagtcctgcacaagatggaatctgatcttgaaggatacaaaaagacctttaccaaaggcccattcattgactacgaaaagcagtcaagcctctccatctatgaggcctgggtcaagatctgggagaagaactcttgggaagaaagaaagaagtacccttttcagcagcttgttagagatgaactggagcgggcggttgcctactacaaacaagattcactctctgaagcggtaaaagtgctaagacaggagctcaacaagcaaaaagcgctaaaggaaaaagaggacctctctcaactggagcgggactacagaacccgaaaggcgaatctcgagatgaaagtacaatccgagcttgatcaagcgggaagtgctttgcctccattggtcagtccaacgccagagcaatggcttgaacgtgccacaagactggttacgcaagcaattgctgataaaaagcagctgcagaccacaaacaatactcttatcaagaattccccaacccctctagaaaagcagaaagccatctacaatggtgagctacttgtggatgagatagccagtctacaggcccgcttagttaagctgaacggaggaggaggatcacaaatttcacaagcgggtatcaacttaattaagagctttgagggtttacaactgaaagcatataaagctgttccgactgagaagcattacaccattggttacggtcattacggttccgatgtttcacctaggcaggttatcactgctaaacaggctgaagacatgttgcgtgatgatgtgcaggcttttgtggatggtgtaaataaagcattaaaagtatctgtcacccaaaatcaatttgatgcacttgtctcattcgcttacaacgttgggttaggggctttcaggtcttcttctctactggaatacttgaatgaaggaagaacagctctagcggcggctgaattccctaaatggaataagtcaggcggtaaagtttatcaagggttgattaaccgtagagcacaggagcaagccttgtttaatagtggaacacctaaaaatgtttaa

SEQ ID NO: 18 - protein, 454 aa, Artificial Sequence
  Protein; Theoretical pI/Mw: 8.71 / 51160.99
MSNDNEVPGSMVIVAQGPDDQYAYEVPPIDSAAVAGNMFGDLIQREIYLQKNIYYPVRSIFEQGTKEKKEINKKVSDQVDGLLKQITQGKREATRQERVDVMSAVLHKMESDLEGYKKTFTKGPFIDYEKQSSLSIYEAWVKIWEKNSWEERKKYPFQQLVRDELERAVAYYKQDSLSEAVKVLRQELNKQKALKEKEDLSQLERDYRTRKANLEMKVQSELDQAGSALPPLVSPTPEQWLERATRLVTQAIADKKQLQTTNNTLIKNSPTPLEKQKAIYNGELLVDEIASLQARLVKLNGGGGSQISQAGINLIKSFEGLQLKAYKAVPTEKHYTIGYGHYGSDVSPRQVITAKQAEDMLRDDVQAFVDGVNKALKVSVTQNQFDALVSFAYNVGLGAFRSSSLLEYLNEGRTALAAAEFPKWNKSGGKVYQGLINRRAQEQALFNSGTPKNV

SEQ ID NO: 19 - DNA, 1404 bp, Artificial Sequence
  P626: S5 TD-RD-Link-BP7e: 1422 bases
atgtccaatgacaacgaagtacctggttccatggttattgtcgcacaaggtccagacgatcaatacgcatacgaggttccccctatcgatagcgcggccgttgccgggaatatgtttggcgacttaattcaaagagaaatatatctacagaaaaacatttattatccagtccgatctatttttgaacaaggaacaaaagaaaagaaggagatcaacaagaaagtatctgatcaagtcgatggcttgctaaagcagatcactcaaggaaaaagggaggccacaaggcaagagcgagtcgatgtcatgtcggcagtcctgcacaagatggaatctgatcttgaaggatacaaaaagacctttaccaaaggcccattcattgactacgaaaagcagtcaagcctctccatctatgaggcctgggtcaagatctgggagaagaactcttgggaagaaagaaagaagtacccttttcagcagcttgttagagatgaactggagcgggcggttgcctactacaaacaagattcactctctgaagcggtaaaagtgctaagacaggagctcaacaagcaaaaagcgctaaaggaaaaagaggacctctctcaactggagcgggactacagaacccgaaaggcgaatctcgagatgaaagtacaatccgagcttgatcaagcgggaagtgctttgcctccattggtcagtccaacgccagagcaatggcttgaacgtgccacaagactggttacgcaagcaattgctgataaaaagcagctgcagaccacaaacaatactcttatcaagaattccccaacccctctagaaaagcagaaagccatctacaatggtgagctacttgtggatgagatagccagtctacaggcccgcttagttaagctgaacggaggaggaggatcaggtgacatttttgatatgctgcgccaagacgaaggcctggacctgaacctgtataaagacacggaaggctactggacgattggtattggtcagctggtcaccaaaaacccgagtaaagatgtggcacgtgctgaactggacaaactgatgggtcgtgtgtgcaatggccgcattacgatggcggaagccgaacaactgtttaaccgtagcgttgaaaatgcacgtcgcgctatcctgcgcaacccgaaactgaaaccggtgtatgatgttctggacgaagtgcgtcgctgtgcgctgatcaacatggtttttcagatgggcgaagcgggtgtcgccggcttcaccaatagcctgcgtatgctgcagcaaaaacgctggaacgatgcggccgtcaatctggcacagtctcgctggtacaaacaaacgccgaatcgtgcgaaacgcgttattgctaccttcaaaacgggcacctgggcggcgtatcgttga

SEQ ID NO: 20 - protein, 467 aa, Artificial Sequence
  Protein; Theoretical pI/Mw: 9.05 / 53373.88
MSNDNEVPGSMVIVAQGPDDQYAYEVPPIDSAAVAGNMFGDLIQREIYLQKNIYYPVRSIFEQGTKEKKEINKKVSDQVDGLLKQITQGKREATRQERVDVMSAVLHKMESDLEGYKKTFTKGPFIDYEKQSSLSIYEAWVKIWEKNSWEERKKYPFQQLVRDELERAVAYYKQDSLSEAVKVLRQELNKQKALKEKEDLSQLERDYRTRKANLEMKVQSELDQAGSALPPLVSPTPEQWLERATRLVTQAIADKKQLQTTNNTLIKNSPTPLEKQKAIYNGELLVDEIASLQARLVKLNGGGGSGDIFDMLRQDEGLDLNLYKDTEGYWTIGIGQLVTKNPSKDVARAELDKLMGRVCNGRITMAEAEQLFNRSVENARRAILRNPKLKPVYDVLDEVRRCALINMVFQMGEAGVAGFTNSLRMLQQKRWNDAAVNLAQSRWYKQTPNRAKRVIATFKTGTWAAYR

SEQ ID NO: 21 - DNA, 1515 bp, Artificial Sequence
  P638: S5 Pyocin with 6X-His tag: 1497 bases
atgtccaatgacaacgaagtacctggttccatggttattgtcgcacaaggtccagacgatcaatacgcatacgaggttccccctatcgatagcgcggccgttgccgggaatatgtttggcgacttaattcaaagagaaatatatctacagaaaaacatttattatccagtccgatctatttttgaacaaggaacaaaagaaaagaaggagatcaacaagaaagtatctgatcaagtcgatggcttgctaaagcagatcactcaaggaaaaagggaggccacaaggcaagagcgagtcgatgtcatgtcggcagtcctgcacaagatggaatctgatcttgaaggatacaaaaagacctttaccaaaggcccattcattgactacgaaaagcagtcaagcctctccatctatgaggcctgggtcaagatctgggagaagaactcttgggaagaaagaaagaagtacccttttcagcagcttgttagagatgaactggagcgggcggttgcctactacaaacaagattcactctctgaagcggtaaaagtgctaagacaggagctcaacaagcaaaaagcgctaaaggaaaaagaggacctctctcaactggagcgggactacagaacccgaaaggcgaatctcgagatgaaagtacaatccgagcttgatcaagcgggaagtgctttgcctccattggtcagtccaacgccagagcaatggcttgaacgtgccacaagactggttacgcaagcaattgctgataaaaagcagctgcagaccacaaacaatactcttatcaagaattccccaacccctctagaaaagcagaaagccatctacaatggtgagctacttgtggatgagatagccagtctacaggcccgcttagttaagctgaacgccgaaacgacacgacgcaggacagaagcagaacgcaaggcggccgaggaacaagcgttgcaagatgctattaaatttactgccgacttttataaggaagtaactgagaaatttggcgcacgaacatcggagatggcgcgccaactggccgaaggcgccagggggaaaaatatcaggagttcggcggaagcaatcaagtcgtttgaaaagcacaaggatgcgttaaataaaaaacttagccttaaagataggcaagccattgccaaagcctttgattctctagacaagcagatgatggcgaagagccttgagaaatttagcaaaggctttggagttgtaggcaaagctattgacgccgccagcctgtaccaagagttcaagatatctacggaaaccggggactggaaaccattctttgtaaaaattgaaacactagctgctggtgcggccgccagttggcttgtgggtattgcatttgccacggcaacagccactcctataggcattctggggttcgcactggtaatggcagttaccggggcgatgattgacgaagaccttctagaaaaagcaaacaatcttgtaatatccattcaccaccaccaccaccactaa

SEQ ID NO: 22 - protein, 504 aa, Artificial Sequence
  Theoretical pI/Mw: 8.50 / 56075.04
MSNDNEVPGSMVIVAQGPDDQYAYEVPPIDSAAVAGNMFGDLIQREIYLQKNIYYPVRSIFEQGTKEKKEINKKVSDQVDGLLKQITQGKREATRQERVDVMSAVLHKMESDLEGYKKTFTKGPFIDYEKQSSLSIYEAWVKIWEKNSWEERKKYPFQQLVRDELERAVAYYKQDSLSEAVKVLRQELNKQKALKEKEDLSQLERDYRTRKANLEMKVQSELDQAGSALPPLVSPTPEQWLERATRLVTQAIADKKQLQTTNNTLIKNSPTPLEKQKAIYNGELLVDEIASLQARLVKLNAETTRRRTEAERKAAEEQALQDAIKFTADFYKEVTEKFGARTSEMARQLAEGARGKNIRSSAEAIKSFEKHKDALNKKLSLKDRQAIAKAFDSLDKQMMAKSLEKFSKGFGVVGKAIDAASLYQEFKISTETGDWKPFFVKIETLAAGAAASWLVGIAFATATATPIGILGFALVMAVTGAMIDEDLLEKANNLVISIHHHHHH

SEQ ID NO: 23 - DNA, 1497 bp, Artificial Sequence
  P652: S5 Pyocin without His tag: 1497 bases
atgtccaatgacaacgaagtacctggttccatggttattgtcgcacaaggtccagacgatcaatacgcatacgaggttccccctatcgatagcgcggccgttgccgggaatatgtttggcgacttaattcaaagagaaatatatctacagaaaaacatttattatccagtccgatctatttttgaacaaggaacaaaagaaaagaaggagatcaacaagaaagtatctgatcaagtcgatggcttgctaaagcagatcactcaaggaaaaagggaggccacaaggcaagagcgagtcgatgtcatgtcggcagtcctgcacaagatggaatctgatcttgaaggatacaaaaagacctttaccaaaggcccattcattgactacgaaaagcagtcaagcctctccatctatgaggcctgggtcaagatctgggagaagaactcttgggaagaaagaaagaagtacccttttcagcagcttgttagagatgaactggagcgggcggttgcctactacaaacaagattcactctctgaagcggtaaaagtgctaagacaggagctcaacaagcaaaaagcgctaaaggaaaaagaggacctctctcaactggagcgggactacagaacccgaaaggcgaatctcgagatgaaagtacaatccgagcttgatcaagcgggaagtgctttgcctccattggtcagtccaacgccagagcaatggcttgaacgtgccacaagactggttacgcaagcaattgctgataaaaagcagctgcagaccacaaacaatactcttatcaagaattccccaacccctctagaaaagcagaaagccatctacaatggtgagctacttgtggatgagatagccagtctacaggcccgcttagttaagctgaacgccgaaacgacacgacgcaggacagaagcagaacgcaaggcggccgaggaacaagcgttgcaagatgctattaaatttactgccgacttttataaggaagtaactgagaaatttggcgcacgaacatcggagatggcgcgccaactggccgaaggcgccagggggaaaaatatcaggagttcggcggaagcaatcaagtcgtttgaaaagcacaaggatgcgttaaataaaaaacttagccttaaagataggcaagccattgccaaagcctttgattctctagacaagcagatgatggcgaagagccttgagaaatttagcaaaggctttggagttgtaggcaaagctattgacgccgccagcctgtaccaagagttcaagatatctacggaaaccggggactggaaaccattctttgtaaaaattgaaacactagctgctggtgcggccgccagttggcttgtgggtattgcatttgccacggcaacagccactcctataggcattctggggttcgcactggtaatggcagttaccggggcgatgattgacgaagaccttctagaaaaagcaaacaatcttgtaatatccatttaa

SEQ ID NO: 24 - protein, 498 aa, Artificial Sequence
  Theoretical pI/Mw: 8.50 / 56075.04
MSNDNEVPGSMVIVAQGPDDQYAYEVPPIDSAAVAGNMFGDLIQREIYLQKNIYYPVRSIFEQGTKEKKEINKKVSDQVDGLLKQITQGKREATRQERVDVMSAVLHKMESDLEGYKKTFTKGPFIDYEKQSSLSIYEAWVKIWEKNSWEERKKYPFQQLVRDELERAVAYYKQDSLSEAVKVLRQELNKQKALKEKEDLSQLERDYRTRKANLEMKVQSELDQAGSALPPLVSPTPEQWLERATRLVTQAIADKKQLQTTNNTLIKNSPTPLEKQKAIYNGELLVDEIASLQARLVKLNAETTRRRTEAERKAAEEQALQDAIKFTADFYKEVTEKFGARTSEMARQLAEGARGKNIRSSAEAIKSFEKHKDALNKKLSLKDRQAIAKAFDSLDKQMMAKSLEKFSKGFGVVGKAIDAASLYQEFKISTETGDWKPFFVKIETLAAGAAASWLVGIAFATATATPIGILGFALVMAVTGAMIDEDLLEKANNLVISI

SEQ ID NO: 25 - DNA, 990 bp, Artificial Sequence
  Fyu A BD- T4 lysozyme fusion
atgagcgacacgatggttgtgaatggcagcggcggcgttccggcgttcctgtttagcggcagcaccctgagcagctatcgtccgaatttcgaggcgaacagcatcaccattgcgctgccgcactatgtggacctgccgggccgtagcaacttcaagctgatgtatatcatgggttttccgattgacaccgagatggaaaaggatagcgagtacagcaacaaaatccgtcaagaaagcaagattagcaaaaccgagggcaccgtgagctacgaacagaaaatcaccgttgagaccggccaagaaaaggatggtgtgaaagtttatcgtgtgatggttctggagggcaccatcgcggagagcattgaacacctggacaagaaagagaacgaagacatcctgaacaacaaccgtaaccgtattgtgctggcggacaacaccgttatcaacttcgataacattagccagctgaaggaatttctgcgtcgtagcgtgaacatcgttattttcgagatgctgcgtatcgacgaacgtctgcgtctgaagatttataaagataccgagggctactataccatcggtattggccacctgctgaccaaaagcccgagcctgaacgcggcgaagagcgaactggacaaagcgatcggccgtaactgcaacggtgtgattaccaaggatgaggcggaaaaactgtttaaccaggacgtggatgcggcggttcgtggtatcctgcgtaacgcgaagctgaaaccggtgtacgacagcctggatgcggttcgtcgttgcgcgctgattaacatggtgttccaaatgggcgagaccggcgttgcgggttttaccaacagcctgcgtatgctgcagcaaaagcgttgggacgaagcggcggttaacctggcgaaaagcatctggtataaccagaccccgaaccgtgcgaaacgtgtgattaccaccttccgtaccggcacctgggatgcgtataaaaacctgtaa

SEQ ID NO: 26 - protein, 329 aa, Artificial Sequence
  Amino acid sequence encoded by SEQ ID NO: 25
MSDTMVVNGSGGVPAFLFSGSTLSSYRPNFEANSITIALPHYVDLPGRSNFKLMYIMGFPIDTEMEKDSEYSNKIRQESKISKTEGTVSYEQKITVETGQEKDGVKVYRVMVLEGTIAESIEHLDKKENEDILNNNRNRIVLADNTVINFDNISQLKEFLRRSVNIVIFEMLRIDERLRLKIYKDTEGYYTIGIGHLLTKSPSLNAAKSELDKAIGRNCNGVITKDEAEKLFNQDVDAAVRGILRNAKLKPVYDSLDAVRRCALINMVFQMGETGVAGFTNSLRMLQQKRWDEAAVNLAKSIWYNQTPNRAKRVITTFRTGTWDAYKNL

SEQ ID NO: 27 - DNA, 1152 bp, Artificial Sequence
  Fyu A BD -GP36 fusion
atgagcgacacgatggttgtgaatggcagcggcggcgttccggcgttcctgtttagcggcagcaccctgagcagctatcgtccgaatttcgaggcgaacagcatcaccattgcgctgccgcactatgtggacctgccgggccgtagcaacttcaagctgatgtatatcatgggttttccgattgacaccgagatggaaaaggatagcgagtacagcaacaaaatccgtcaagaaagcaagattagcaaaaccgagggcaccgtgagctacgaacagaaaatcaccgttgagaccggccaagaaaaggatggtgtgaaagtttatcgtgtgatggttctggagggcaccatcgcggagagcattgaacacctggacaagaaagagaacgaagacatcctgaacaacaaccgtaaccgtattgtgctggcggacaacaccgttatcaacttcgataacattagccagctgaaggaatttctgcgtcgtagcgtgaacatcgttggtgtggccctggaccgcacgcgggttgatccccaggcagtcggcaacgaggtgctcaagcgcaacgcggataagctgaatgcgatgcggggcgccgagtacggtgccaacgtcaaggtcagcggcacggacattcgcatgaacgggggtaacagtgccggcatgctgaagcaggacgtgttcaactggcggaaggaactggctcagttcgaggcttaccgaggggaggcgtataaggatgccgatggttatagtgtgggcctggggcattacctgggcagtggcaatgctggggcaggtactacagtcacgcctgagcaagccgcgcagtggttcgccgaggacaccgaccgcgcactcgaccagggtgtgaggttggccgacgagctgggcgttacgaacaatgcctctatcctgggattggccggtatggccttccagatgggcgaaggacgtgcccggcagttccgtaacaccttccaggcgatcaaggatcgcaacaaggaagccttcgaggctggtgtgcgaaacagcaagtggtacacgcagacgcccaaccgggccgaggcattcatcaagcgcatggcgccccacttcgatacaccgagtcaaatcggtgtcgattggtacagcgccgcaacagcggagtga

SEQ ID NO: 28 - protein, 383 aa, Artificial Sequence
  Amino acid sequence encoded by SEQ ID NO: 27
MSDTMVVNGSGGVPAFLFSGSTLSSYRPNFEANSITIALPHYVDLPGRSNFKLMYIMGFPIDTEMEKDSEYSNKIRQESKISKTEGTVSYEQKITVETGQEKDGVKVYRVMVLEGTIAESIEHLDKKENEDILNNNRNRIVLADNTVINFDNISQLKEFLRRSVNIVGVALDRTRVDPQAVGNEVLKRNADKLNAMRGAEYGANVKVSGTDIRMNGGNSAGMLKQDVFNWRKELAQFEAYRGEAYKDADGYSVGLGHYLGSGNAGAGTTVTPEQAAQWFAEDTDRALDQGVRLADELGVTNNASILGLAGMAFQMGEGRARQFRNTFQAIKDRNKEAFEAGVRNSKWYTQTPNRAEAFIKRMAPHFDTPSQIGVDWYSAATAE

SEQ ID NO: 29 - DNA, 1955 bp, Artificial Sequence
  pelB-FyuA receptor: 2028 bases
atgaaatacctgctgccgaccgctgctgctggtctgctgctcctcgctgcccagccggcgatggccatgggccagacttcacagcaagacgaaagcacgctggtggttaccgccagtaaacaatcttcccgctcggcatcagccaacaacgtctcgtctactgttgtcagcgcgccggaattaagcgacgccggcgtcaccgccagcgacaaactccccagagtcttgcccgggctcaatattgaaaatagcggcaacatgcttttttcgacgatctcgctacgcggcgtctcttcagcgcaggacttctataaccccgccgtcaccctgtatgtcgatggcgtccctcagctttccaccaacaccatccaggcgcttaccgatgtgcaaagcgtggagttgctgcgaggcccacagggaacgttatatggcaaaagcgctcagggcgggatcatcaacatcgtcacccagcagccggacagcacgccgcgcggctatattgaaggcggcgtcagtagccgcgacagttatcgaagtaagttcaacctgagcggccccattcaggatggcctgctgtacggcagcgtcaccctgttacgccaggttgatgacggcgacatgattaaccccgcgacgggaagcgatgacttaggcggcacccgcgccagcatagggaatgtgaaactgcgtctggcgccggacgatcagccctgggaaatgggctttgccgcctcacgcgaatgtacccgcgccacccaggacgcctatgtgggatggaatgatattaagggccgtaagctgtcgatcagcgatggttcaccagacccgtacatgcggcgctgcactgacagccagaccctgagtgggaaatacaccaccgatgactgggttttcaacctgatcagcgcctggcagcagcagcattattcgcgcaccttcccttccggttcgttaatcgtcaatatgcctcagcgctggaatcaggatgtgcaggagctgcgcgccgcaaccctgggcgatgcgcgtaccgttgatatggtgtttgggctgtaccggcagaacacccgcgagaagttaaattcagcctacgacatgccgacaatgccttatttaagcagtaccggctataccaccgctgaaacgctggccgcatacagtgacctgacctggcatttaaccgatcgttttgatatcggcggcggcgtgcgcttctcgcatgataaatccagtacacaatatcacggcagcatgctcggcaacccgtttggcgaccagggtaagagcaatgacgatcaggtgctcgggcagctatccgcaggctatatgctgaccgatgactggagagtgtatacccgtgtagcccagggatataaaccttccgggtacaacatcgtgcctactgcgggtcttgatgccaaaccgttcgtcgccgagaaatccatcaactatgaacttggcacccgctacgaaaccgctgacgtcacgctgcaagccgcgacgttttatacccacaccaaagacatgcagctttactctggcccggtcgggatgcagacattaagcaatgcgggtaaagccgacgccaccggcgttgagcttgaagcgaagtggcggtttgcgccaggctggtcatgggatatcaatggcaacgtgatccgttccgaattcaccaatgacagtgagttgtatcacggtaaccgggtgccgttcgtaccacgttatggcgcgggaagcagcgtgaacggtgtgattgatacgcgctatggcgcactgatgccccgactggcggttaatctggtcgggccgcattatttcgatggcgacaaccagttgcggcaaggcacctatgccaccctggacagcagcctgggctggcaggcaacggcagcagcgccgtcgcgcaggtcaatatgggtcgcaccgtcggtatcaatacgcgaattgatttcttctga

SEQ ID NO: 30 - protein, 675 aa, Artificial Sequence
  Theoretical pI/Mw: 5.35 / 73772.10
MKYLLPTAAAGLLLLAAQPAMAMGQTSQQDESTLVVTASKQSSRSASANNVSSTVVSAPELSDAGVTASDKLPRVLPGLNIENSGNMLFSTISLRGVSSAQDFYNPAVTLYVDGVPQLSTNTIQALTDVQSVELLRGPQGTLYGKSAQGGIINIVTQQPDSTPRGYIEGGVSSRDSYRSKFNLSGPIQDGLLYGSVTLLRQVDDGDMINPATGSDDLGGTRASIGNVKLRLAPDDQPWEMGFAASRECTRATQDAYVGWNDIKGRKLSISDGSPDPYMRRCTDSQTLSGKYTTDDWVFNLISAWQQQHYSRTFPSGSLIVNMPQRWNQDVQELRAATLGDARTVDMVFGLYRQNTREKLNSAYDMPTMPYLSSTGYTTAETLAAYSDLTWHLTDRFDIGGGVRFSHDKSSTQYHGSMLGNPFGDQGKSNDDQVLGQLSAGYMLTDDWRVYTRVAQGYKPSGYNIVPTAGLDAKPFVAEKSINYELGTRYETADVTLQAATFYTHTKDMQLYSGPVGMQTLSNAGKADATGVELEAKWRFAPGWSWDINGNVIRSEFTNDSELYHGNRVPFVPRYGAGSSVNGVIDTRYGALMPRLAVNLVGPHYFDGDNQLRQGTYATLDSSLGWQATERMNISVYVDNLFDRRYRTYGYMNGSSAVAQVNMGRTVGINTRIDFF